European Patent Application EP 4 137 587 A1, published February 22, 2023. Title: Metodo di screening di un acaro di Demodex spp. Applicant: Ingeno S.r.l. Application EP. The sequence listing filed with the application follows.

SEQUENCE LISTING (15 sequences)

SEQ ID NO: 1 - DNA, 21 bp, synthetic construct
  source 1..21: mol_type = other DNA
tgctgcggtattttgactgtg

SEQ ID NO: 2 - DNA, 20 bp, synthetic construct
  source 1..20: mol_type = other DNA
ttgctgcggtattttgactg

SEQ ID NO: 3 - DNA, 20 bp
tttggggtcttctcgtcttt

SEQ ID NO: 4 - DNA, 20 bp, synthetic construct
  source 1..20: mol_type = other DNA
ttttggggtcttctcgtctt

SEQ ID NO: 5 - DNA, 21 bp, synthetic construct
  source 1..21: mol_type = other DNA
ggggtcttctcgtctttagga

SEQ ID NO: 6 - DNA, 21 bp, synthetic construct
  source 1..21: mol_type = other DNA
aaaatcaatctttcccccaaa

SEQ ID NO: 7 - DNA, 21 bp, synthetic construct
  source 1..21: mol_type = other DNA
aaagattttggggtcttctcg

SEQ ID NO: 8 - DNA, 20 bp, synthetic construct
  source 1..20: mol_type = other DNA
gattttggggtcttctcgtc

SEQ ID NO: 9 - DNA, 21 bp, synthetic construct
  source 1..21: mol_type = other DNA
gattttggggtcttctcgtct

SEQ ID NO: 10 - DNA, 21 bp, synthetic construct
  source 1..21: mol_type = other DNA
agattttggggtcttctcgtc

SEQ ID NO: 11 - DNA, 21 bp, synthetic construct
  source 1..21: mol_type = other DNA
tggggtcttctcgtctttagg

SEQ ID NO: 12 - DNA, 22 bp, synthetic construct
  source 1..22: mol_type = other DNA
  modified_base 21: mod_base = OTHER; note = n is an abasic site or t
  modified_base 22: mod_base = OTHER; note = n is an abasic site or g
  modified_base 1: mod_base = OTHER; note = n is an abasic site or t
ntgctgcggtattttgactgnn

SEQ ID NO: 13 - DNA, 22 bp, synthetic construct
  source 1..22: mol_type = other DNA
  modified_base 1: mod_base = OTHER; note = n is an abasic site or t
  modified_base 2: mod_base = OTHER; note = n is an abasic site or t
  modified_base 22: mod_base = OTHER; note = n is an abasic site or t
nntttggggtcttctcgtcttn

SEQ ID NO: 14 - DNA, 24 bp, synthetic construct
  source 1..24: mol_type = other DNA
  modified_base 1: mod_base = OTHER; note = n is an abasic site or a
  modified_base 2: mod_base = OTHER; note = n is an abasic site or a
  modified_base 3: mod_base = OTHER; note = n is an abasic site or a
  modified_base 22: mod_base = OTHER; note = n is an abasic site or t
  modified_base 23: mod_base = OTHER; note = n is an abasic site or c
  modified_base 24: mod_base = OTHER; note = n is an abasic site or t
nnngattttggggtcttctcgnnn

SEQ ID NO: 15 - DNA, 22 bp, synthetic construct
  source 1..22: mol_type = other DNA
  modified_base 1: mod_base = OTHER; note = n is an abasic site or t
  modified_base 22: mod_base = OTHER; note = n is an abasic site or a
nggggtcttctcgtctttaggn